European Patent Application EP 4 393 956 A1, published July 3, 2024. Title: Novel anti-MUC1 antibodies and uses thereof. Applicant: 펩트론. Application KR. The sequence listing filed with the application follows.

SEQUENCE LISTING (6 sequences)

SEQ ID NO: 1 - protein, 10 aa, synthetic construct
  REGION 1..10: note = MUC1 Heavy chain CDR1
GYTFTSYWMH

SEQ ID NO: 2 - protein, 17 aa, synthetic construct
  REGION 1..17: note = MUC1 Heavy chain CDR2
YINPGTGYIEYNQKFKD

SEQ ID NO: 3 - protein, 7 aa, synthetic construct
  REGION 1..7: note = MUC1 Heavy chain CDR3
STAPFDY

SEQ ID NO: 4 - protein, 11 aa, synthetic construct
  REGION 1..11: note = MUC1 Light chain CDR1
  SITE 1: note = MISC_FEATURE - X is the residue being substituted.
  SITE 7: note = MISC_FEATURE - X is the residue being substituted.
XASQDIXSYLS

SEQ ID NO: 5 - protein, 7 aa, synthetic construct
  REGION 1..7: note = MUC1 Light chain CDR2
YATRLAD

SEQ ID NO: 6 - protein, 9 aa, synthetic construct
  REGION 1..9: note = MUC1 Light chain CDR3
LQYDESPYT